European Patent Application EP 4 596 573 A1, published August 6, 2025. Title: A fusion protein that forms self-assembly comprising a peptide tag in which major amino acids are composed of charged and polar amino acids, and a method for purifying recombinant protein using the same. Applicant: CCRIPO Inc. Application KR. The sequence listing filed with the application follows.

SEQUENCE LISTING (82 sequences)

SEQ ID NO: 1 - protein, 6 aa, synthetic construct
  REGION 1..6: note = His6 tag_AA
HHHHHH

SEQ ID NO: 2 - protein, 15 aa, synthetic construct
  REGION 1..15: note = P(SE)2 tag_AA
PSESEPSESEPSESE

SEQ ID NO: 3 - protein, 27 aa, synthetic construct
  REGION 1..27: note = P(SE)4 tag_AA
PSESESESEPSESESESEPSESESESE

SEQ ID NO: 4 - protein, 21 aa, synthetic construct
  REGION 1..21: note = P(SE)2IA tag_AA
PSESEIAPSESEIAPSESEIA

SEQ ID NO: 5 - protein, 18 aa, synthetic construct
  REGION 1..18: note = PSEIAH tag_AA
PSEIAHPSEIAHPSEIAH

SEQ ID NO: 6 - protein, 16 aa, synthetic construct
  REGION 1..16: note = PS(E)6 tag_AA
PSEEEEEEPSEEEEEE

SEQ ID NO: 7 - protein, 12 aa, synthetic construct
  REGION 1..12: note = PS(E)10 tag_AA
PSEEEEEEEEEE

SEQ ID NO: 8 - protein, 12 aa, synthetic construct
  REGION 1..12: note = PS(D)10 tag_AA
PSDDDDDDDDDD

SEQ ID NO: 9 - protein, 25 aa, synthetic construct
  REGION 1..25: note = SHD tag_AA
SSHHDHHDHHSSPSSHHDHHDHHSS

SEQ ID NO: 10 - protein, 19 aa, synthetic construct
  REGION 1..19: note = EctP1 tag_AA
SSRSSSHRRHDHHDHRRGS

SEQ ID NO: 11 - protein, 10 aa, synthetic construct
  REGION 1..10: note = His6 clone_AA
MDPMHHHHHH

SEQ ID NO: 12 - protein, 25 aa, synthetic construct
  REGION 1..25: note = His6:P(SE)2 clone_AA
MDPMHHHHHHPSESEPSESEPSESE

SEQ ID NO: 13 - protein, 36 aa, synthetic construct
  REGION 1..36: note = His6:P(SE)4 clone_AA
MDPMHHHHHHPSESESESEPSESESESEPSESESES

SEQ ID NO: 14 - protein, 31 aa, synthetic construct
  REGION 1..31: note = His6:P(SE)2IA clone_AA
MDPMHHHHHHPSESEIAPSESEIAPSESEIA

SEQ ID NO: 15 - protein, 28 aa, synthetic construct
  REGION 1..28: note = His6:PSEIAH clone_AA
MDPMHHHHHHPSEIAHPSEIAHPSEIAH

SEQ ID NO: 16 - protein, 26 aa, synthetic construct
  REGION 1..26: note = His6:PS(E)6 clone_AA
MDPMHHHHHHPSEEEEEEPSEEEEEE

SEQ ID NO: 17 - protein, 22 aa, synthetic construct
  REGION 1..22: note = His6:PS(E)10 clone_AA
MDPMHHHHHHPSEEEEEEEEEE

SEQ ID NO: 18 - protein, 22 aa, synthetic construct
  REGION 1..22: note = His6:PS(D)10 clone_AA
MDPMHHHHHHPSDDDDDDDDDD

SEQ ID NO: 19 - protein, 31 aa, synthetic construct
  REGION 1..31: note = His6:EctP1 clone_AA
MDPMHHHHHHPGSSRSSSHRRHDHHDHRRGS

SEQ ID NO: 20 - protein, 36 aa, synthetic construct
  REGION 1..36: note = His6:SHD clone_AA
MDPMHHHHHHPSSHHDHHDHHSSPSSHHDHHDHHSS

SEQ ID NO: 21 - protein, 19 aa, synthetic construct
  REGION 1..19: note = P(SE)2 clone_AA
MDPMPSESEPSESEPSESE

SEQ ID NO: 22 - protein, 31 aa, synthetic construct
  REGION 1..31: note = P(SE)4 clone_AA
MDPMPSESESESEPSESESESEPSESESESE

SEQ ID NO: 23 - protein, 20 aa, synthetic construct
  REGION 1..20: note = P(SE)6 clone_AA
MDPMPSEEEEEEPSEEEEEE

SEQ ID NO: 24 - protein, 21 aa, synthetic construct
  REGION 1..21: note = EctP1 clone_AA
MGSSRSSSHRRHDHHDHRRGS

SEQ ID NO: 25 - protein, 29 aa, synthetic construct
  REGION 1..29: note = SHD clone_AA
MDPMSSHHDHHDHHSSPSSHHDHHDHHSS

SEQ ID NO: 26 - protein, 217 aa, synthetic construct
  REGION 1..217: note = His6:P(SE)2:INF-a2 clone_AA
MDPMHHHHHHPSESEPSESEPSESEGTGSPPVPSTPPTPSPSCRSENLYFQGCDLPQTHSLGSRRTLMLLAQMRRISLFSCLKDRHDFGFPQEEFGNQFQKAETIPVLHEMIQQIFNLFSTKDSSAAWDETLLDKFYTELYQQLNDLEACVIQGVGVTETPLMKEDSILAVRKYFQRITLYLKEKKYSPCAWEVVRAEIMRSFSLSTNLQESLRSKE

SEQ ID NO: 27 - protein, 281 aa, synthetic construct
  REGION 1..281: note = His6:P(SE)2:TEV protease clone_AA
MDPMHHHHHHPSESEPSESEPSESEGTGSPPVPSTPPTPSPSCRSGESLFKGPRDYNPISSTICHLTNESDGHTTSLYGIGFGPFIITNKHLFRRNNGTLLVQSLHGVFKVKNTTTLQQHLIDGRDMIIIRMPKDFPPFPQKLKFREPQREERICLVTTNFQTKSMSSMVSDTSCTFPSSDGIFWKHWIQTKDGQCGSPLVSTRDGFIVGIHSASNFTNTNNYFTSVPKNFMELLTNQEAQQWVSGWRLNADSVLWGGHKVFMVKPEEPFQPVKEATQLMN

SEQ ID NO: 28 - protein, 266 aa, synthetic construct
  REGION 1..266: note = His6:P(SE)2:HER LC clone_AA
MDPMHHHHHHPSESEPSESEPSESEGTGSPPVPSTPPTPSPSCRSENLYFQGDIQMTQSPSSLSASVGDRVTITCRASQDVNTAVAWYQQKPGKAPKLLIYSASFLYSGVPSRFSGSRSGTDFTLTISSLQPEDFATYYCQQHYTTPPTFGQGTKVEIKRTVAAPSVFIFPPSDEQLKSGTASVVCLLNNFYPREAKVQWKVDNALQSGNSQESVTEQDSKDSTYSLSSTLTLSKADYEKHKVYACEVTHQGLSSPVTKSFNRGEC

SEQ ID NO: 29 - protein, 293 aa, synthetic construct
  REGION 1..293: note = His6:P(SE)4:TEV protease clone_AA
MDPMHHHHHHPSESESESEPSESESESEPSESESESEGTGSPPVPSTPPTPSPSCRSGESLFKGPRDYNPISSTICHLTNESDGHTTSLYGIGFGPFIITNKHLFRRNNGTLLVQSLHGVFKVKNTTTLQQHLIDGRDMIIIRMPKDFPPFPQKLKFREPQREERICLVTTNFQTKSMSSMVSDTSCTFPSSDGIFWKHWIQTKDGQCGSPLVSTRDGFIVGIHSASNFTNTNNYFTSVPKNFMELLTNQEAQQWVSGWRLNADSVLWGGHKVFMVKPEEPFQPVKEATQLMN

SEQ ID NO: 30 - protein, 278 aa, synthetic construct
  REGION 1..278: note = His6:P(SE)4:HER LC clone_AA
MDPMHHHHHHPSESESESEPSESESESEPSESESESEGTGSPPVPSTPPTPSPSCRSENLYFQGDIQMTQSPSSLSASVGDRVTITCRASQDVNTAVAWYQQKPGKAPKLLIYSASFLYSGVPSRFSGSRSGTDFTLTISSLQPEDFATYYCQQHYTTPPTFGQGTKVEIKRTVAAPSVFIFPPSDEQLKSGTASVVCLLNNFYPREAKVQWKVDNALQSGNSQESVTEQDSKDSTYSLSSTLTLSKADYEKHKVYACEVTHQGLSSPVTKSFNRGEC

SEQ ID NO: 31 - protein, 235 aa, synthetic construct
  REGION 1..235: note = His6:P(SE)2IA:rhG-CSF clone_AA
MDPMHHHHHHPSESEIAPSESEIAPSESEIAGTGSPPVPSTPPTPSPSCRSAAAENLYFQGTPLGPASSLPQSFLLKCLEQVRKIQGDGAALQEKLCATYKLCHPEELVLLGHSLGIPWAPLSSCPSQALQLAGCLSQLHSGLFLYQGLLQALEGISPELGPTLDTLQLDVADFATTIWQQMEELGMAPALQPTQGAMPAFASAFQRRAGGVLVASHLQSFLEVSYRVLRHLAQP

SEQ ID NO: 32 - protein, 232 aa, synthetic construct
  REGION 1..232: note = His6:PSEIAH:rhG-CSF clone_AA
MDPMHHHHHHPSEIAHPSEIAHPSEIAHGTGSPPVPSTPPTPSPSCRSAAAENLYFQGTPLGPASSLPQSFLLKCLEQVRKIQGDGAALQEKLCATYKLCHPEELVLLGHSLGIPWAPLSSCPSQALQLAGCLSQLHSGLFLYQGLLQALEGISPELGPTLDTLQLDVADFATTIWQQMEELGMAPALQPTQGAMPAFASAFQRRAGGVLVASHLQSFLEVSYRVLRHLAQP

SEQ ID NO: 33 - protein, 223 aa, synthetic construct
  REGION 1..223: note = His6:EctP1:INF-a2 clone_AA
MDPMHHHHHHPGSSRSSSHRRHDHHDHRRGSGTGSPPVPSTPPTPSPSCRSENLYFQGCDLPQTHSLGSRRTLMLLAQMRRISLFSCLKDRHDFGFPQEEFGNQFQKAETIPVLHEMIQQIFNLFSTKDSSAAWDETLLDKFYTELYQQLNDLEACVIQGVGVTETPLMKEDSILAVRKYFQRITLYLKEKKYSPCAWEVVRAEIMRSFSLSTNLQESLRSKE

SEQ ID NO: 34 - protein, 287 aa, synthetic construct
  REGION 1..287: note = His6:EctP1:TEV protease clone_AA
MDPMHHHHHHPGSSRSSSHRRHDHHDHRRGSGTGSPPVPSTPPTPSPSCRSGESLFKGPRDYNPISSTICHLTNESDGHTTSLYGIGFGPFIITNKHLFRRNNGTLLVQSLHGVFKVKNTTTLQQHLIDGRDMIIIRMPKDFPPFPQKLKFREPQREERICLVTTNFQTKSMSSMVSDTSCTFPSSDGIFWKHWIQTKDGQCGSPLVSTRDGFIVGIHSASNFTNTNNYFTSVPKNFMELLTNQEAQQWVSGWRLNADSVLWGGHKVFMVKPEEPFQPVKEATQLMN

SEQ ID NO: 35 - protein, 228 aa, synthetic construct
  REGION 1..228: note = His6:SHD:INF-a2 clone_AA
MDPMHHHHHHPSSHHDHHDHHSSPSSHHDHHDHHSSGTGSPPVPSTPPTPSPSCRSENLYFQGCDLPQTHSLGSRRTLMLLAQMRRISLFSCLKDRHDFGFPQEEFGNQFQKAETIPVLHEMIQQIFNLFSTKDSSAAWDETLLDKFYTELYQQLNDLEACVIQGVGVTETPLMKEDSILAVRKYFQRITLYLKEKKYSPCAWEVVRAEIMRSFSLSTNLQESLRSKE

SEQ ID NO: 36 - protein, 233 aa, synthetic construct
  REGION 1..233: note = SHD:rhG-CSF clone_AA
MDPMSSHHDHHDHHSSPSSHHDHHDHHSSGTGSPPVPSTPPTPSPSCRSAAAENLYFQGTPLGPASSLPQSFLLKCLEQVRKIQGDGAALQEKLCATYKLCHPEELVLLGHSLGIPWAPLSSCPSQALQLAGCLSQLHSGLFLYQGLLQALEGISPELGPTLDTLQLDVADFATTIWQQMEELGMAPALQPTQGAMPAFASAFQRRAGGVLVASHLQSFLEVSYRVLRHLAQP

SEQ ID NO: 37 - protein, 221 aa, synthetic construct
  REGION 1..221: note = SHD:INF-a2 clone_AA
MDPMSSHHDHHDHHSSPSSHHDHHDHHSSGTGSPPVPSTPPTPSPSCRSENLYFQGCDLPQTHSLGSRRTLMLLAQMRRISLFSCLKDRHDFGFPQEEFGNQFQKAETIPVLHEMIQQIFNLFSTKDSSAAWDETLLDKFYTELYQQLNDLEACVIQGVGVTETPLMKEDSILAVRKYFQRITLYLKEKKYSPCAWEVVRAEIMRSFSLSTNLQESLRSKE

SEQ ID NO: 38 - protein, 285 aa, synthetic construct
  REGION 1..285: note = SHD:TEV protease clone_AA
MDPMSSHHDHHDHHSSPSSHHDHHDHHSSGTGSPPVPSTPPTPSPSCRSGESLFKGPRDYNPISSTICHLTNESDGHTTSLYGIGFGPFIITNKHLFRRNNGTLLVQSLHGVFKVKNTTTLQQHLIDGRDMIIIRMPKDFPPFPQKLKFREPQREERICLVTTNFQTKSMSSMVSDTSCTFPSSDGIFWKHWIQTKDGQCGSPLVSTRDGFIVGIHSASNFTNTNNYFTSVPKNFMELLTNQEAQQWVSGWRLNADSVLWGGHKVFMVKPEEPFQPVKEATQLMN

SEQ ID NO: 39 - protein, 229 aa, synthetic construct
  REGION 1..229: note = His6:P(SE)4:INF-a2 clone_AA
MDPMHHHHHHPSESESESEPSESESESEPSESESESEGTGSPPVPSTPPTPSPSCRSENLYFQGCDLPQTHSLGSRRTLMLLAQMRRISLFSCLKDRHDFGFPQEEFGNQFQKAETIPVLHEMIQQIFNLFSTKDSSAAWDETLLDKFYTELYQQLNDLEACVIQGVGVTETPLMKEDSILAVRKYFQRITLYLKEKKYSPCAWEVVRAEIMRSFSLSTNLQESLRSKE

SEQ ID NO: 40 - protein, 237 aa, synthetic construct
  REGION 1..237: note = GFP clone_AA
SKGEELFTGVVPILVELDGDVNGHKFSVSGEGEGDATYGKLTLKFICTTGKLPVPWPTLVTTFSYGVQCFSRYPDHMKRHDFFKSAMPEGYVQERTIFFKDDGNYKTRAEVKFEGDTLVNRIELKGIDFKEDGNILGHKLEYNYNSHNVYIMADKQKNGIKANFKTRHNIEDGGVQLADHYQQNTPIGDGPVLLPDNHYLSTQSALSKDPNEKRDHMVLLEFVTAAGITHGMDELYK

SEQ ID NO: 41 - protein, 16 aa, synthetic construct
  REGION 1..16: note = Hinge_AA
GSPPVPSTPPTPSPSC

SEQ ID NO: 42 - DNA, 18 bp, synthetic construct
  misc_feature 1..18: note = His6 tag_NT
  source 1..18: mol_type = other DNA
catcaccatcaccaccat

SEQ ID NO: 43 - DNA, 45 bp, synthetic construct
  misc_feature 1..45: note = P(SE)2 tag_NT
  source 1..45: mol_type = other DNA
ccaagcgagagtgaacctagtgaaagcgagcctagcgagagtgaa

SEQ ID NO: 44 - DNA, 81 bp, synthetic construct
  misc_feature 1..81: note = P(SE)4 tag_NT
  source 1..81: mol_type = other DNA
ccaagcgagagtgaaagcgagagtgagcctagtgaaagcgagagtgaaagcgaaccgagcgagagcgaaagtgagagcgag

SEQ ID NO: 45 - DNA, 63 bp, synthetic construct
  misc_feature 1..63: note = P(SE)2IA tag_NT
  source 1..63: mol_type = other DNA
ccaagcgagagtgaaattgctcctagtgaaagcgagatagcacctagcgagagtgaaatcgct

SEQ ID NO: 46 - DNA, 54 bp, synthetic construct
  misc_feature 1..54: note = PSEIAH tag_NT
  source 1..54: mol_type = other DNA
ccaagtgagattgctcatcctagcgaaatagcacacccaagtgagatagcacat

SEQ ID NO: 47 - DNA, 48 bp, synthetic construct
  misc_feature 1..48: note = PS(E)6 tag_NT
  source 1..48: mol_type = other DNA
ccaagcgaggaggaagaagaggaacctagtgaagaggaggaggaagag

SEQ ID NO: 48 - DNA, 36 bp, synthetic construct
  misc_feature 1..36: note = PS(E)10 tag_NT
  source 1..36: mol_type = other DNA
ccaagcgaggaggaagaagaggaagaagaggaggag

SEQ ID NO: 49 - DNA, 36 bp, synthetic construct
  misc_feature 1..36: note = PS(D)10 tag_NT
  source 1..36: mol_type = other DNA
ccaagcgatgacgacgatgatgacgatgacgacgac

SEQ ID NO: 50 - DNA, 75 bp, synthetic construct
  misc_feature 1..75: note = SHD tag_NT
  source 1..75: mol_type = other DNA
tctagccaccatgatcatcatgaccaccactctagcccatcgtcacatcacgaccaccacgatcatcattcgtct

SEQ ID NO: 51 - DNA, 57 bp, synthetic construct
  misc_feature 1..57: note = EctP1 tag_NT
  source 1..57: mol_type = other DNA
tctagccgcagcagcagccatcgccgccatgatcatcatgatcatcgccgcggcagc

SEQ ID NO: 52 - DNA, 30 bp, synthetic construct
  misc_feature 1..30: note = His6 clone_NT
  source 1..30: mol_type = other DNA
atggatccaatgcatcaccatcaccaccat

SEQ ID NO: 53 - DNA, 75 bp, synthetic construct
  misc_feature 1..75: note = His6:P(SE)2 clone_NT
  source 1..75: mol_type = other DNA
atggatccaatgcatcaccatcaccatcacccaagcgagagtgaacctagtgaaagcgagcctagcgagagtgaa

SEQ ID NO: 54 - DNA, 111 bp, synthetic construct
  misc_feature 1..111: note = His6:P(SE)4 clone_NT
  source 1..111: mol_type = other DNA
atggatccaatgcatcaccatcaccatcacccaagcgagagtgaaagcgagagtgagcctagtgaaagcgagagtgaaagcgaaccgagcgagagcgaaagtgagagcgag

SEQ ID NO: 55 - DNA, 93 bp, synthetic construct
  misc_feature 1..93: note = His6:P(SE)2IA clone_NT
  source 1..93: mol_type = other DNA
atggatccaatgcatcaccatcaccatcacccaagcgagagtgaaattgctcctagtgaaagcgagatagcacctagcgagagtgaaatcgct

SEQ ID NO: 56 - DNA, 84 bp, synthetic construct
  misc_feature 1..84: note = His6:PSEIAH clone_NT
  source 1..84: mol_type = other DNA
atggatccaatgcatcaccatcaccaccatccaagtgagattgctcatcctagcgaaatagcacacccaagtgagatagcacat

SEQ ID NO: 57 - DNA, 78 bp, synthetic construct
  misc_feature 1..78: note = His6:PS(E)6 clone_NT
  source 1..78: mol_type = other DNA
atggatccaatgcatcaccatcaccatcacccaagcgaggaggaagaagaggaacctagtgaagaggaggaggaagag

SEQ ID NO: 58 - DNA, 66 bp, synthetic construct
  misc_feature 1..66: note = His6:PS(E)10 clone_NT
  source 1..66: mol_type = other DNA
atggatccaatgcatcaccatcaccatcacccaagcgaggaggaagaagaggaagaagaggaggag

SEQ ID NO: 59 - DNA, 66 bp, synthetic construct
  misc_feature 1..66: note = His6:PS(D)10 clone_NT
  source 1..66: mol_type = other DNA
atggatccaatgcatcaccatcaccatcacccaagcgatgacgacgatgatgacgatgacgacgac

SEQ ID NO: 60 - DNA, 93 bp, synthetic construct
  misc_feature 1..93: note = His6:EctP1 clone_NT
  source 1..93: mol_type = other DNA
atggatccaatgcatcaccatcaccaccatcctggttctagccgcagcagcagccatcgccgccatgatcatcatgatcatcgccgcggcagc

SEQ ID NO: 61 - DNA, 108 bp, synthetic construct
  misc_feature 1..108: note = His6:SHD clone_NT
  source 1..108: mol_type = other DNA
atggatccaatgcatcaccatcaccaccatccttctagccaccatgatcatcatgaccaccactctagcccatcgtcacatcacgaccaccacgatcatcattcgtct

SEQ ID NO: 62 - DNA, 108 bp, synthetic construct; identical to SEQ ID NO: 61
  misc_feature 1..108: note = P(SE)2 clone_NT
  source 1..108: mol_type = other DNA

SEQ ID NO: 63 - DNA, 93 bp, synthetic construct
  misc_feature 1..93: note = P(SE)4 clone_NT
  source 1..93: mol_type = other DNA
atggatccaatgccaagcgagagtgaaagcgagagtgagcctagtgaaagcgagagtgaaagcgaaccgagcgagagcgaaagtgagagcgag

SEQ ID NO: 64 - DNA, 60 bp, synthetic construct
  misc_feature 1..60: note = P(SE)6 clone_NT
  source 1..60: mol_type = other DNA
atggatccaatgccaagcgaggaggaagaagaggaacctagtgaagaggaggaggaagag

SEQ ID NO: 65 - DNA, 63 bp, synthetic construct
  misc_feature 1..63: note = EctP1 clone_NT
  source 1..63: mol_type = other DNA
atgggttctagccgcagcagcagccatcgccgccatgatcatcatgatcatcgccgcggcagc

SEQ ID NO: 66 - DNA, 87 bp, synthetic construct
  misc_feature 1..87: note = SHD clone_NT
  source 1..87: mol_type = other DNA
atggatccaatgtctagccaccatgatcatcatgaccaccactctagcccatcgtcacatcacgaccaccacgatcatcattcgtct

SEQ ID NO: 67 - DNA, 654 bp, synthetic construct
  misc_feature 1..654: note = His6:P(SE)2:INF-a2 clone_NT
  source 1..654: mol_type = other DNA
atggatccaatgcatcaccatcaccatcacccaagcgagagtgaacctagtgaaagcgagcctagcgagagtgaaggtaccggttctccaccagtaccaagcacacctccaactccgagtccgagttgtagatctgaaaacctgtattttcagggctgcgatctcccacaaacccactccttaggttctcgacgtactctaatgcttctcgctcagatgaggaggatttcacttttcagttgtttgaaggatcgtcacgacttcggatttccccaagaagagtttggaaaccaattccaaaaggctgagacaattccagttttgcacgaaatgattcaacaaatctttaatctgtttagcactaaggatagcagcgcagcatgggatgaaacactccttgataaattttatacagaattatatcagcaactgaatgaccttgaggcatgcgtcatacagggtgttggggtaacagagactcctctcatgaaagaagacagtattttagccgttcgtaaatattttcagcgtattactctttatcttaaagaaaaaaaatactccccttgcgcatgggaggttgtccgagcagaaattatgaggagcttctccctctctacaaatctgcaagagtctttgagaagtaaagaatga

SEQ ID NO: 68 - DNA, 846 bp, synthetic construct
  misc_feature 1..846: note = His6:P(SE)2:TEV protease clone_NT
  source 1..846: mol_type = other DNA
atggatccaatgcatcaccatcaccatcacccaagcgagagtgaacctagtgaaagcgagcctagcgagagtgaaggtaccggttctccaccagtaccaagcacacctccaactccgagtccgagttgtagatctggagaaagcttgtttaaggggccgcgtgattacaacccgatatcgagcaccatttgtcatttgacgaatgaatctgatgggcacacaacatcgttgtatggtattggatttggtcccttcatcattacaaacaagcacttgtttagaagaaataatggaacactgttggtccaatcactacatggtgtattcaaggtcaagaacaccacgactttgcaacaacacctcattgatgggagggacatgataattattcgcatgcctaaggatttcccaccatttcctcaaaagctgaaatttagagagccacaaagggaagagcgcatatgtcttgtgacaaccaacttccaaactaagagcatgtctagcatggtgtcagacactagttgcacattcccttcatctgatggcatattctggaagcattggattcaaaccaaggatgggcagtgtggcagtccattagtatcaactagagatgggttcattgttggtatacactcagcatcgaatttcaccaacacaaacaattatttcacaagcgtgccgaaaaacttcatggaattgttgacaaatcaggaggcgcagcagtgggttagtggttggcgattaaatgctgactcagtattgtgggggggccataaagttttcatggtgaaacctgaagagccttttcagccagttaaggaagcgactcaacttatgaattaa

SEQ ID NO: 69 - DNA, 801 bp, synthetic construct
  misc_feature 1..801: note = His6:P(SE)2:HER LC clone_NT
  source 1..801: mol_type = other DNA
atggatccaatgcatcaccatcaccatcacccaagcgagagtgaacctagtgaaagcgagcctagcgagagtgaaggtaccggttctccaccagtaccaagcacacctccaactccgagtccgagttgtagatctgaaaacctgtattttcagggcgatattcagatgacacagagccctagtagtctgagcgctagcgtgggagatagagtgacaattacatgtagagccagccaggatgtgaacacagccgtggcttggtaccagcagaagcctggcaaggcccccaagcttctgatctattccgcttctttcctctactctggggtccccagcaggtttagcgggagcaggagcgggaccgactttacccttacaatcagctccctgcagcccgaggacttcgccacatactactgccagcagcattacactactccacccactttcgggcaaggaactaaagtggagattaagcggacagtggccgcccccagcgtgttcattttccccccctccgacgagcagctgaagagcggcacagccagcgtggtgtgcctgctgaacaacttctacccacgggaggccaaggtgcagtggaaggtggacaacgctctgcagagcggcaacagccaggaaagcgtgaccgagcaggattccaaggatagcacatacagcctgtcgagcaccctgacactgagcaaggccgactacgagaagcacaaggtgtacgcctgcgaggtgacacaccaggggctcagcagccccgtcacaaagagcttcaacaggggggagtgctag

SEQ ID NO: 70 - DNA, 882 bp, synthetic construct
  misc_feature 1..882: note = His6:P(SE)4:TEV protease clone_NT
  source 1..882: mol_type = other DNA
atggatccaatgcatcaccatcaccatcacccaagcgagagtgaaagcgagagtgagcctagtgaaagcgagagtgaaagcgaaccgagcgagagcgaaagtgagagcgagggtaccggttctccaccagtaccaagcacacctccaactccgagtccgagttgtagatctggagaaagcttgtttaaggggccgcgtgattacaacccgatatcgagcaccatttgtcatttgacgaatgaatctgatgggcacacaacatcgttgtatggtattggatttggtcccttcatcattacaaacaagcacttgtttagaagaaataatggaacactgttggtccaatcactacatggtgtattcaaggtcaagaacaccacgactttgcaacaacacctcattgatgggagggacatgataattattcgcatgcctaaggatttcccaccatttcctcaaaagctgaaatttagagagccacaaagggaagagcgcatatgtcttgtgacaaccaacttccaaactaagagcatgtctagcatggtgtcagacactagttgcacattcccttcatctgatggcatattctggaagcattggattcaaaccaaggatgggcagtgtggcagtccattagtatcaactagagatgggttcattgttggtatacactcagcatcgaatttcaccaacacaaacaattatttcacaagcgtgccgaaaaacttcatggaattgttgacaaatcaggaggcgcagcagtgggttagtggttggcgattaaatgctgactcagtattgtgggggggccataaagttttcatggtgaaacctgaagagccttttcagccagttaaggaagcgactcaacttatgaattaa

SEQ ID NO: 71 - DNA, 837 bp, synthetic construct
  misc_feature 1..837: note = His6:P(SE)4:HER LC clone_NT
  source 1..837: mol_type = other DNA
atggatccaatgcatcaccatcaccatcacccaagcgagagtgaaagcgagagtgagcctagtgaaagcgagagtgaaagcgaaccgagcgagagcgaaagtgagagcgagggtaccggttctccaccagtaccaagcacacctccaactccgagtccgagttgtagatctgaaaacctgtattttcagggcgatattcagatgacacagagccctagtagtctgagcgctagcgtgggagatagagtgacaattacatgtagagccagccaggatgtgaacacagccgtggcttggtaccagcagaagcctggcaaggcccccaagcttctgatctattccgcttctttcctctactctggggtccccagcaggtttagcgggagcaggagcgggaccgactttacccttacaatcagctccctgcagcccgaggacttcgccacatactactgccagcagcattacactactccacccactttcgggcaaggaactaaagtggagattaagcggacagtggccgcccccagcgtgttcattttccccccctccgacgagcagctgaagagcggcacagccagcgtggtgtgcctgctgaacaacttctacccacgggaggccaaggtgcagtggaaggtggacaacgctctgcagagcggcaacagccaggaaagcgtgaccgagcaggattccaaggatagcacatacagcctgtcgagcaccctgacactgagcaaggccgactacgagaagcacaaggtgtacgcctgcgaggtgacacaccaggggctcagcagccccgtcacaaagagcttcaacaggggggagtgctag

SEQ ID NO: 72 - DNA, 708 bp, synthetic construct
  misc_feature 1..708: note = His6:P(SE)2IA:rhG-CSF clone_NT
  source 1..708: mol_type = other DNA
atggatccaatgcatcaccatcaccatcacccaagcgagagtgaaattgctcctagtgaaagcgagatagcacctagcgagagtgaaatcgctggtaccggttctccaccagtaccaagcacacctccaactccgagtccgagttgtagatctgcggccgcagaaaacctgtattttcagggcacccccctgggccctgccagctccctgccccagagcttcctgctcaagtgcttagagcaagtgaggaagatccagggcgatggcgcagcgctccaggagaagctgtgtgccacctacaagctgtgccaccccgaggagctggtgctgctcggacactctctgggcatcccctgggctcccctgagcagctgccccagccaggccctacagctggcaggctgcttgagccaactccatagcggccttttcctctaccaggggctcctacaggccctggaagggatctcccccgagttgggtcccaccttggacacactacagctggacgtcgccgactttgccaccaccatctggcagcagatggaagaactgggaatggcccctgccctacagcccacccagggtgccatgccggccttcgcctctgctttccagcgccgggcaggaggggtcctagttgcctcccatctacagagcttcctggaggtgtcgtaccgcgttctacgccaccttgcccagccctga

SEQ ID NO: 73 - DNA, 699 bp, synthetic construct
  misc_feature 1..699: note = His6:PSEIAH:rhG-CSF clone_NT
  source 1..699: mol_type = other DNA
atggatccaatgcatcaccatcaccaccatccaagtgagattgctcatcctagcgaaatagcacacccaagtgagatagcacatggtaccggttctccaccagtaccaagcacacctccaactccgagtccgagttgtagatctgcggccgcagaaaacctgtattttcagggcacccccctgggccctgccagctccctgccccagagcttcctgctcaagtgcttagagcaagtgaggaagatccagggcgatggcgcagcgctccaggagaagctgtgtgccacctacaagctgtgccaccccgaggagctggtgctgctcggacactctctgggcatcccctgggctcccctgagcagctgccccagccaggccctacagctggcaggctgcttgagccaactccatagcggccttttcctctaccaggggctcctacaggccctggaagggatctcccccgagttgggtcccaccttggacacactacagctggacgtcgccgactttgccaccaccatctggcagcagatggaagaactgggaatggcccctgccctacagcccacccagggtgccatgccggccttcgcctctgctttccagcgccgggcaggaggggtcctagttgcctcccatctacagagcttcctggaggtgtcgtaccgcgttctacgccaccttgcccagccctga

SEQ ID NO: 74 - DNA, 672 bp, synthetic construct
  misc_feature 1..672: note = His6:EctP1:INF-a2 clone_NT
  source 1..672: mol_type = other DNA
atggatccaatgcatcaccatcaccaccatcctggttctagccgcagcagcagccatcgccgccatgatcatcatgatcatcgccgcggcagcggtaccggttctccaccagtaccaagcacacctccaactccgagtccgagttgtagatctgaaaacctgtattttcagggctgcgatctcccacaaacccactccttaggttctcgacgtactctaatgcttctcgctcagatgaggaggatttcacttttcagttgtttgaaggatcgtcacgacttcggatttccccaagaagagtttggaaaccaattccaaaaggctgagacaattccagttttgcacgaaatgattcaacaaatctttaatctgtttagcactaaggatagcagcgcagcatgggatgaaacactccttgataaattttatacagaattatatcagcaactgaatgaccttgaggcatgcgtcatacagggtgttggggtaacagagactcctctcatgaaagaagacagtattttagccgttcgtaaatattttcagcgtattactctttatcttaaagaaaaaaaatactccccttgcgcatgggaggttgtccgagcagaaattatgaggagcttctccctctctacaaatctgcaagagtctttgagaagtaaagaatga

SEQ ID NO: 75 - DNA, 864 bp, synthetic construct
  misc_feature 1..864: note = His6:EctP1:TEV protease clone_NT
  source 1..864: mol_type = other DNA
atggatccaatgcatcaccatcaccaccatcctggttctagccgcagcagcagccatcgccgccatgatcatcatgatcatcgccgcggcagcggtaccggttctccaccagtaccaagcacacctccaactccgagtccgagttgtagatctggagaaagcttgtttaaggggccgcgtgattacaacccgatatcgagcaccatttgtcatttgacgaatgaatctgatgggcacacaacatcgttgtatggtattggatttggtcccttcatcattacaaacaagcacttgtttagaagaaataatggaacactgttggtccaatcactacatggtgtattcaaggtcaagaacaccacgactttgcaacaacacctcattgatgggagggacatgataattattcgcatgcctaaggatttcccaccatttcctcaaaagctgaaatttagagagccacaaagggaagagcgcatatgtcttgtgacaaccaacttccaaactaagagcatgtctagcatggtgtcagacactagttgcacattcccttcatctgatggcatattctggaagcattggattcaaaccaaggatgggcagtgtggcagtccattagtatcaactagagatgggttcattgttggtatacactcagcatcgaatttcaccaacacaaacaattatttcacaagcgtgccgaaaaacttcatggaattgttgacaaatcaggaggcgcagcagtgggttagtggttggcgattaaatgctgactcagtattgtgggggggccataaagttttcatggtgaaacctgaagagccttttcagccagttaaggaagcgactcaacttatgaattaa

SEQ ID NO: 76 - DNA, 687 bp, synthetic construct
  misc_feature 1..687: note = His6:SHD:INF-a2 clone_NT
  source 1..687: mol_type = other DNA
atggatccaatgcatcaccatcaccaccatccttctagccaccatgatcatcatgaccaccactctagcccatcgtcacatcacgaccaccacgatcatcattcgtctggtaccggttctccaccagtaccaagcacacctccaactccgagtccgagttgtagatctgaaaacctgtattttcagggctgcgatctcccacaaacccactccttaggttctcgacgtactctaatgcttctcgctcagatgaggaggatttcacttttcagttgtttgaaggatcgtcacgacttcggatttccccaagaagagtttggaaaccaattccaaaaggctgagacaattccagttttgcacgaaatgattcaacaaatctttaatctgtttagcactaaggatagcagcgcagcatgggatgaaacactccttgataaattttatacagaattatatcagcaactgaatgaccttgaggcatgcgtcatacagggtgttggggtaacagagactcctctcatgaaagaagacagtattttagccgttcgtaaatattttcagcgtattactctttatcttaaagaaaaaaaatactccccttgcgcatgggaggttgtccgagcagaaattatgaggagcttctccctctctacaaatctgcaagagtctttgagaagtaaagaatga

SEQ ID NO: 77 - DNA, 702 bp, synthetic construct
  misc_feature 1..702: note = SHD:rhG-CSF clone_NT
  source 1..702: mol_type = other DNA
atggatccaatgtctagccaccatgatcatcatgaccaccactctagcccatcgtcacatcacgaccaccacgatcatcattcgtctggtaccggttctccaccagtaccaagcacacctccaactccgagtccgagttgtagatctgcggccgcagaaaacctgtattttcagggcacccccctgggccctgccagctccctgccccagagcttcctgctcaagtgcttagagcaagtgaggaagatccagggcgatggcgcagcgctccaggagaagctgtgtgccacctacaagctgtgccaccccgaggagctggtgctgctcggacactctctgggcatcccctgggctcccctgagcagctgccccagccaggccctacagctggcaggctgcttgagccaactccatagcggccttttcctctaccaggggctcctacaggccctggaagggatctcccccgagttgggtcccaccttggacacactacagctggacgtcgccgactttgccaccaccatctggcagcagatggaagaactgggaatggcccctgccctacagcccacccagggtgccatgccggccttcgcctctgctttccagcgccgggcaggaggggtcctagttgcctcccatctacagagcttcctggaggtgtcgtaccgcgttctacgccaccttgcccagccctga

SEQ ID NO: 78 - DNA, 666 bp, synthetic construct
  misc_feature 1..666: note = SHD:INF-a2 clone_NT
  source 1..666: mol_type = other DNA
atggatccaatgtctagccaccatgatcatcatgaccaccactctagcccatcgtcacatcacgaccaccacgatcatcattcgtctggtaccggttctccaccagtaccaagcacacctccaactccgagtccgagttgtagatctgaaaacctgtattttcagggctgcgatctcccacaaacccactccttaggttctcgacgtactctaatgcttctcgctcagatgaggaggatttcacttttcagttgtttgaaggatcgtcacgacttcggatttccccaagaagagtttggaaaccaattccaaaaggctgagacaattccagttttgcacgaaatgattcaacaaatctttaatctgtttagcactaaggatagcagcgcagcatgggatgaaacactccttgataaattttatacagaattatatcagcaactgaatgaccttgaggcatgcgtcatacagggtgttggggtaacagagactcctctcatgaaagaagacagtattttagccgttcgtaaatattttcagcgtattactctttatcttaaagaaaaaaaatactccccttgcgcatgggaggttgtccgagcagaaattatgaggagcttctccctctctacaaatctgcaagagtctttgagaagtaaagaatga

SEQ ID NO: 79 - DNA, 858 bp, synthetic construct
  misc_feature 1..858: note = SHD:TEV protease clone_NT
  source 1..858: mol_type = other DNA
atggatccaatgtctagccaccatgatcatcatgaccaccactctagcccatcgtcacatcacgaccaccacgatcatcattcgtctggtaccggttctccaccagtaccaagcacacctccaactccgagtccgagttgtagatctggagaaagcttgtttaaggggccgcgtgattacaacccgatatcgagcaccatttgtcatttgacgaatgaatctgatgggcacacaacatcgttgtatggtattggatttggtcccttcatcattacaaacaagcacttgtttagaagaaataatggaacactgttggtccaatcactacatggtgtattcaaggtcaagaacaccacgactttgcaacaacacctcattgatgggagggacatgataattattcgcatgcctaaggatttcccaccatttcctcaaaagctgaaatttagagagccacaaagggaagagcgcatatgtcttgtgacaaccaacttccaaactaagagcatgtctagcatggtgtcagacactagttgcacattcccttcatctgatggcatattctggaagcattggattcaaaccaaggatgggcagtgtggcagtccattagtatcaactagagatgggttcattgttggtatacactcagcatcgaatttcaccaacacaaacaattatttcacaagcgtgccgaaaaacttcatggaattgttgacaaatcaggaggcgcagcagtgggttagtggttggcgattaaatgctgactcagtattgtgggggggccataaagttttcatggtgaaacctgaagagccttttcagccagttaaggaagcgactcaacttatgaattaa

SEQ ID NO: 80 - DNA, 690 bp, synthetic construct
  misc_feature 1..690: note = His6:P(SE)4:INF-a2 clone_NT
  source 1..690: mol_type = other DNA
atggatccaatgcatcaccatcaccatcacccaagcgagagtgaaagcgagagtgagcctagtgaaagcgagagtgaaagcgaaccgagcgagagcgaaagtgagagcgagggtaccggttctccaccagtaccaagcacacctccaactccgagtccgagttgtagatctgaaaacctgtattttcagggctgcgatctcccacaaacccactccttaggttctcgacgtactctaatgcttctcgctcagatgaggaggatttcacttttcagttgtttgaaggatcgtcacgacttcggatttccccaagaagagtttggaaaccaattccaaaaggctgagacaattccagttttgcacgaaatgattcaacaaatctttaatctgtttagcactaaggatagcagcgcagcatgggatgaaacactccttgataaattttatacagaattatatcagcaactgaatgaccttgaggcatgcgtcatacagggtgttggggtaacagagactcctctcatgaaagaagacagtattttagccgttcgtaaatattttcagcgtattactctttatcttaaagaaaaaaaatactccccttgcgcatgggaggttgtccgagcagaaattatgaggagcttctccctctctacaaatctgcaagagtctttgagaagtaaagaatga

SEQ ID NO: 81 - DNA, 714 bp, synthetic construct
  misc_feature 1..714: note = GFP clone_NT
  source 1..714: mol_type = other DNA
agtaaaggagaggagttgtttactggtgttgtcccgattttagttgaacttgacggtgatgttaatgggcacaagttctctgtcagtggagaaggggaaggcgatgcaacatatggtaagctcacgttgaagtttatttgcactactggaaaactccctgttccgtggccaacacttgtgactacgttttcttacggtgttcagtgtttttcaagataccctgatcatatgaagcggcacgatttctttaagagcgcgatgcctgagggatacgtgcaggaaagaaccatcttcttcaaggacgacggtaattataagacacgtgctgaagttaagttcgagggagacaccttggtgaatcgaatagaacttaaaggaatcgattttaaggaagatggaaacattctcggccacaagttggagtacaactacaactcacataacgtatacataatggcagataagcaaaagaacggcatcaaggcaaacttcaagaccaggcacaatatcgaggatgggggtgtgcaactagctgatcattatcagcaaaatactccaattggtgatggacctgtcctcttaccagataatcattatctgtccacgcaatctgccctgtcgaaggaccccaacgaaaagagagaccatatggtgcttcttgagttcgtaacagctgctgggattacacatggtatggacgagctatataagtga

SEQ ID NO: 82 - DNA, 48 bp, synthetic construct
  misc_feature 1..48: note = Hinge_NT
  source 1..48: mol_type = other DNA
ggttctccaccagtaccaagcacacctccaactccgagtccgagttgt